European Patent Application EP 4 306 657 A1, published January 17, 2024. Title: Composition for diagnosing pancreatic cancer. Applicant: ACURASYSBIO Co.,Ltd. The sequence listing filed with the application follows.

SEQUENCE LISTING (18 sequences)

SEQ ID NO: 1 - protein, 506 aa, Homo sapiens
MLKPLWKAAVAPTWPCSMPPRRPWDREAGTLQVLGALAVLWLGSVALICLLWQVPRPPTWGQVQPKDVPRSWEHGSSPAWEPLEAEARQQRDSCQLVLVESIPQDLPSAAGSPSAQPLGQAWLQLLDTAQESVHVASYYWSLTGPDIGVNDSSSQLGEALLQKLQQLLGRNISLAVATSSPTLARTSTDLQVLAARGAHVRQVPMGRLTRGVLHSKFWVVDGRHIYMGSANMDWRSLTQVKELGAVIYNCSHLAQDLEKTFQTYWVLGVPKAVLPKTWPQNFSSHFNRFQPFHGLFDGVPTTAYFSASPPALCPQGRTRDLEALLAVMGSAQEFIYASVMEYFPTTRFSHPPRYWPVLDNALRAAAFGKGVRVRLLVGCGLNTDPTMFPYLRSLQALSNPAANVSVDVKVFIVPVGNHSNIPFSRVNHSKFMVTEKAAYIGTSNWSEDYFSSTAGVGLVVTQSPGAQPAGATVQEQLRQLFERDWSSRYAVGLDGQAPGQDCVWQG

SEQ ID NO: 2 - protein, 598 aa, Homo sapiens [sequence omitted]

SEQ ID NO: 3 - protein, 231 aa, Homo sapiens
MQDEERYMTLNVQSKKRSSAQTSQLTFKDYSVTLHWYKILLGISGTVNGILTLTLISLILLVSQGVLLKCQKGSCSNATQYEDTGDLKVNNGTRRNISNKDLCASRSADQTVLCQSEWLKYQGKCYWFSNEMKSWSDSYVYCLERKSHLLIIHDQLEMAFIQKNLRQLNYVWIGLNFTSLKMTWTWVDGSPIDSKIFFIKGPAKENSCAAIKESKIFSETCSSVFKWICQY

SEQ ID NO: 4 - protein, 119 aa, Homo sapiens
MKALSPVRGCYEAVCCLSERSLAIARGRGKGPAAEEPLSLLDDMNHCYSRLRELVPGVPRGTQLSQVEILQRVIDYILDLQVVLAEPAPGPPDGPHLPIQTAELAPELVISNDKRSFCH

SEQ ID NO: 5 - protein, 459 aa, Homo sapiens [sequence omitted]

SEQ ID NO: 6 - DNA, 21 bp, Artificial Sequence
  PLD4 forward primer
caaattctgggttgtggatgg

SEQ ID NO: 7 - DNA, 21 bp, Artificial Sequence
  PLD4 reverse primer
aggtggctgcagttatagatg

SEQ ID NO: 8 - DNA, 18 bp, Artificial Sequence
  NR4A1 forward primer
gacaacgcttcatgccag

SEQ ID NO: 9 - DNA, 21 bp, Artificial Sequence
  NR4A1 reverse primer
ttgttagccaggcagatgtac

SEQ ID NO: 10 - DNA, 21 bp, Artificial Sequence
  KLRF1 forward primer
gaaaaggagttctgcccaaac

SEQ ID NO: 11 - DNA, 22 bp, Artificial Sequence
  KLRF1 reverse primer
agaaaccaacaggatcaaggag

SEQ ID NO: 12 - DNA, 21 bp, Artificial Sequence
  IL7R forward primer
gtagtcatcactccagaaagc

SEQ ID NO: 13 - DNA, 21 bp, Artificial Sequence
  IL7R reverse primer
acctggaagaggagagaatag

SEQ ID NO: 14 - DNA, 21 bp, Artificial Sequence
  ID3 forward primer
gactacattctcgacctgcag

SEQ ID NO: 15 - DNA, 21 bp, Artificial Sequence
  ID3 reverse primer
tcgttggagatgacaagttcc

SEQ ID NO: 16 - DNA, 23 bp, Artificial Sequence
  PLD4-FAM probe
tctgacgcaggtgaaggagcttg

SEQ ID NO: 17 - DNA, 25 bp, Artificial Sequence
  IL7R-FAM probe
cagttggaagtgaatggatcgcagc

SEQ ID NO: 18 - DNA, 22 bp, Artificial Sequence
  ID3-FAM probe
ctcggctgtctggatgggaagg